European Patent Specification EP 3 507 369 B1, published June 12, 2024. Title: ANTI-CD20 ANTIBODY. Applicant: Beijing Mabworks Biotech Co. Ltd. The sequence listing filed with the application follows.

SEQUENCE LISTING (4 sequences)

SEQ ID NO: 1 - protein, 219 aa, Homo sapiens
DIVMTQTPLSLPVTPGEPASISCRSSKSLLHSNGITYLYWYLQKPGQSPQLLIYQMSNLVSGVPDRFSGSGSGTDFTLKISRVEAEDVGVYYCAQNLELPYTFGGGTKVEIKRTVAAPSVFIFPPSDEQLKSGTASVVCLLNNFYPREAKVQWKVDNALQSGNSQESVTEQDSKDSTYSLSSTLTLSKADYEKHKVYACEVTHQGLSSPVTKSFNRGEC

SEQ ID NO: 2 - protein, 444 aa, Homo sapiens
QVQLVQSGAEVKPGSSVVSCKASGYAFSYSWINWVRQAPGQGLEWMGRIFPGDGDTDYNGKFKGRVTITADKSTSTAYMELSSLRSEDTAVYYCARNVFDGYWLVYWGQGTLVTVSSASTKGPSVFPLAPSSKSTSGGTAALGCLVDYFPEPVTVSWNSGALTSGVHTFPAVLQSSGLYSLSSVVTVPSSSLGTQTYICNVNHKPSNTKVDKKVEPKSCDKTHTCPPCPAPELLGGPSVFLFPPKPKDTLMISRTPEVTCVVVDVSHEDPEVFNWYVDGVEVHNAKTKPREEQYNSTYRVVSVLTVLHQDWLNGKEYKCKVSNKALPAPIEKTISKAKGQPREPQVYTLPPSRDELTKNQVSLTCLVGFYPSDIAVEWESNGQPENNYKTTPPVLDSDGSFFLYSKLTVDKSRWQQGNVFSCSVMHEALHNHYTQKSLSLSPGK

SEQ ID NO: 3 - DNA, 657 bp, Homo sapiens
gatatcgtgatgacccagactccactctccctgcccgtcacccctggagagcccgccagcattagctgcaggtctagcaagagcctcttgcacagcaatggcatcacttatttgtattggtacctgcaaaagccagggcagtctccacagctcctgatttatcaaatgtccaaccttgtctctggcgtccctgaccggttctccggatccgggtcaggcactgatttcacactgaaaatcagcagggtggaggctgaggatgttggagtttattactgcgctcagaatctagaacttccttacaccttcggcggagggaccaaggtggagatcaaacgtacggtggctgcaccatctgtcttcatcttcccgccatctgatgagcagttgaaatctggaactgcctctgttgtgtgcctgctgaataacttctatcccagagaggccaaagtacagtggaaggtggataacgccctccaatcgggtaactcccaggagagtgtcacagagcaggacagcaaggacagcacctacagcctcagcagcaccctgacgctgagcaaagcagactacgagaaacacaaagtctacgcctgcgaagtcacccatcagggcctgagctcgcccgtcacaaagagcttcaacaggggagagtgt

SEQ ID NO: 4 - DNA, 1347 bp, Homo sapiens
caggtgcaattggtgcagtctggcgctgaagttaagaagcctgggagttcagtgaaggtctcctgcaaggcttccggatacgccttcagctattcttggatcaattgggtgcggcaggcgcctggacaagggctcgagtggatgggacggatctttcccggcgatggggatactgactacaatgggaaattcaagggcagagtcacaattaccgccgacaaatccactagcacagcctatatggagctgagcagcctgagatctgaggacacggccgtgtattactgtgcaagaaatgtctttgatggttactggcttgtttactggggccagggaaccctggtcaccgtctcctcagctagcaccaagggcccatcggtcttccccctggcaccctcctccaagagcacctctgggggcacagcggccctgggctgcctggtcaaggactacttccccgaaccggtgacggtgtcgtggaactcaggcgccctgaccagcggcgtgcacaccttcccggctgtcctacagtcctcaggactctactccctcagcagcgtggtgactgtgccctctagcagcttgggcacccagacctacatctgcaacgtgaatcacaagcccagcaacaccaaggtggacaagaaagttgagcccaaatcttgtgacaaaactcacacatgcccaccgtgcccagcacctgaactcctggggggaccgtcagtcttcctcttccccccaaaacccaaggacaccctcatgatctcccggacccctgaggtcacatgcgtggtggtggacgtgagccacgaagaccctgaggtcaagttcaactggtacgtggacggcgtggaggtgcataatgccaagacaaagccgcgggaggagcagtacaacagcacgtaccgtgtggtcagcgtcctcaccgtcctgcaccaggactggctgaatggcaaggagtacaagtgcaaggtctccaacaaagccctcccagcccccatcgagaaaaccatctccaaagccaaagggcagccccgagaaccacaggtgtacaccctgcccccatcccgggatgagctgaccaagaaccaggtcagcctgacctgcctggtcaaaggcttctatcccagcgacatcgccgtggagtgggagagcaatgggcagccggagaacaactacaagaccacgcctcccgtgctggactccgacggctccttcttcctctacagcaagctcaccgtggacaagagcaggtggcagcaggggaacgtcttctcatgctccgtgatgcatgaggctctgcacaaccactacacgcagaagagcctctccctgtctccgggtaaa